European Patent Application EP 4 342 541 A2, published March 27, 2024. Title: Antibody Fc variants for Enhanced Serum Half-life. Applicant: Kookmin University Industry Academy Cooperation Foundation. The sequence listing filed with the application follows.

SEQUENCE LISTING (37 sequences)

SEQ ID NO: 1 - DNA, 20 bp, synthetic construct
  misc_feature 1..20: note = pMopac12-seq-Fw
  source 1..20: mol_type = other DNA
ccaggctttacactttatgc

SEQ ID NO: 2 - DNA, 44 bp, synthetic construct
  misc_feature 1..44: note = Fc-M252-1-Rv
  source 1..44: mol_type = other DNA
cctcaggggtccgggagatgwagagggtgtccttgggttttggg

SEQ ID NO: 3 - DNA, 44 bp, synthetic construct
  misc_feature 1..44: note = Fc-M252-2-Rv
  source 1..44: mol_type = other DNA
cctcaggggtccgggagatknbgagggtgtccttgggttttggg

SEQ ID NO: 4 - DNA, 44 bp, synthetic construct
  misc_feature 1..44: note = Fc-M252-3-Rv
  source 1..44: mol_type = other DNA
cctcaggggtccgggagatccagagggtgtccttgggttttggg

SEQ ID NO: 5 - DNA, 19 bp, synthetic construct
  misc_feature 1..19: note = Fc-M428-Fw
  source 1..19: mol_type = other DNA
atctcccggacccctgagg

SEQ ID NO: 6 - DNA, 50 bp, synthetic construct
  misc_feature 1..50: note = Fc-M428-1-Rv
  source 1..50: mol_type = other DNA
gtagtggttgtgcagagcctcatggwacacggagcatgagaagacgttcc

SEQ ID NO: 7 - DNA, 50 bp, synthetic construct
  misc_feature 1..50: note = Fc-M428-2-Rv
  source 1..50: mol_type = other DNA
gtagtggttgtgcagagcctcatgknbcacggagcatgagaagacgttcc

SEQ ID NO: 8 - DNA, 50 bp, synthetic construct
  misc_feature 1..50: note = Fc-M428-3-Rv
  source 1..50: mol_type = other DNA
gtagtggttgtgcagagcctcatgccacacggagcatgagaagacgttcc

SEQ ID NO: 9 - DNA, 24 bp, synthetic construct
  misc_feature 1..24: note = Fc-M428-frg3-Fw
  source 1..24: mol_type = other DNA
catgaggctctgcacaaccactac

SEQ ID NO: 10 - DNA, 19 bp, synthetic construct
  misc_feature 1..19: note = pMopac12-seq-Rv
  source 1..19: mol_type = other DNA
ctgcccatgttgacgattg

SEQ ID NO: 11 - DNA, 22 bp, synthetic construct
  misc_feature 1..22: note = Fc-Sub#0-Rv
  source 1..22: mol_type = other DNA
gtccttgggttttggggggaag

SEQ ID NO: 12 - DNA, 59 bp, synthetic construct
  misc_feature 1..59: note = Fc-Sub#1-1-Fw
  source 1..59: mol_type = other DNA
cttccccccaaaacccaaggacnnkctcatgatctcccggacccctgaggtcacatgcg

SEQ ID NO: 13 - DNA, 59 bp, synthetic construct
  misc_feature 1..59: note = Fc-Sub#1-2-Fw
  source 1..59: mol_type = other DNA
cttccccccaaaacccaaggacaccnnkatgatctcccggacccctgaggtcacatgcg

SEQ ID NO: 14 - DNA, 59 bp, synthetic construct
  misc_feature 1..59: note = Fc-Sub#1-3-Fw
  source 1..59: mol_type = other DNA
cttccccccaaaacccaaggacaccctcatgnnktcccggacccctgaggtcacatgcg

SEQ ID NO: 15 - DNA, 59 bp, synthetic construct
  misc_feature 1..59: note = Fc-Sub#1-4-Fw
  source 1..59: mol_type = other DNA
cttccccccaaaacccaaggacaccctcatgatcnnkcggacccctgaggtcacatgcg

SEQ ID NO: 16 - DNA, 59 bp, synthetic construct
  misc_feature 1..59: note = Fc-Sub#1-5-Fw
  source 1..59: mol_type = other DNA
cttccccccaaaacccaaggacaccctcatgatctccnnkacccctgaggtcacatgcg

SEQ ID NO: 17 - DNA, 19 bp, synthetic construct
  misc_feature 1..19: note = Fc-Sub#1-Rv
  source 1..19: mol_type = other DNA
gacggtgaggacgctgacc

SEQ ID NO: 18 - DNA, 62 bp, synthetic construct
  misc_feature 1..62: note = Fc-Sub#2-1-Fw
  source 1..62: mol_type = other DNA
ggtcagcgtcctcaccgtcnnkcaccaggactggctgaatggcaaggagtacaagtgcaagg

SEQ ID NO: 19 - DNA, 62 bp, synthetic construct
  misc_feature 1..62: note = Fc-Sub#2-2-Fw
  source 1..62: mol_type = other DNA
ggtcagcgtcctcaccgtcctgcacnnkgactggctgaatggcaaggagtacaagtgcaagg

SEQ ID NO: 20 - DNA, 62 bp, synthetic construct
  misc_feature 1..62: note = Fc-Sub#2-3-Fw
  source 1..62: mol_type = other DNA
ggtcagcgtcctcaccgtcctgcaccaggactggnnkaatggcaaggagtacaagtgcaagg

SEQ ID NO: 21 - DNA, 23 bp, synthetic construct
  misc_feature 1..23: note = Fc-Sub#2-Rv
  source 1..23: mol_type = other DNA
cacggagcatgagaagacgttcc

SEQ ID NO: 22 - DNA, 71 bp, synthetic construct
  misc_feature 1..71: note = Fc-Sub#3-1-Fw
  source 1..71: mol_type = other DNA
ggaacgtcttctcatgctccgtgctgcatnnkgctctgcacaaccactacacgcagaagagcctctccctg

SEQ ID NO: 23 - DNA, 71 bp, synthetic construct
  misc_feature 1..71: note = Fc-Sub#3-2-Fw
  source 1..71: mol_type = other DNA
ggaacgtcttctcatgctccgtgctgcatgaggctnnkcacaaccactacacgcagaagagcctctccctg

SEQ ID NO: 24 - DNA, 71 bp, synthetic construct
  misc_feature 1..71: note = Fc-Sub#3-3-Fw
  source 1..71: mol_type = other DNA
ggaacgtcttctcatgctccgtgctgcatgaggctctgcacnnkcactacacgcagaagagcctctccctg

SEQ ID NO: 25 - DNA, 71 bp, synthetic construct
  misc_feature 1..71: note = Fc-Sub#3-4-Fw
  source 1..71: mol_type = other DNA
ggaacgtcttctcatgctccgtgctgcatgaggctctgcacaaccacnnkacgcagaagagcctctccctg

SEQ ID NO: 26 - DNA, 16 bp, synthetic construct
  misc_feature 1..16: note = ep-Fc-Fw
  source 1..16: mol_type = other DNA
ccagccggccatggcg

SEQ ID NO: 27 - DNA, 21 bp, synthetic construct
  misc_feature 1..21: note = ep-Fc-Rv
  source 1..21: mol_type = other DNA
gaattcggcccccgaggcccc

SEQ ID NO: 28 - protein, 227 aa, Homo sapiens
DKTHTCPPCPAPELLGGPSVFLFPPKPKDTLMISRTPEVTCVVVDVSHEDPEVKFNWYVDGVEVHNAKTKPREEQYNSTYRVVSVLTVLHQDWLNGKEYKCKVSNKALPAPIEKTISKAKGQPREPQVYTLPPSRDELTKNQVSLTCLVKGFYPSDIAVEWESNGQPENNYKTTPPVLDSDGSFFLYSKLTVDKSRWQQGNVFSCSVMHEALHNHYTQKSLSLSPGK

SEQ ID NO: 29 - DNA, 681 bp, Homo sapiens
  source 1..681: mol_type = genomic DNA
gacaaaactcacacatgcccaccgtgcccagcacctgaactcctggggggaccgtcagtcttcctcttccccccaaaacccaaggacaccctcatgatctcccggacccctgaggtcacatgcgtggtggtggacgtgagccacgaagaccctgaggtcaagttcaactggtacgtggacggcgtggaggtgcataatgccaagacaaagccgcgggaggagcagtacaacagcacgtaccgtgtggtcagcgtcctcaccgtcctgcaccaggactggctgaatggcaaggagtacaagtgcaaggtctccaacaaagccctcccagcccccatcgagaaaaccatctccaaagccaaagggcagccccgagaaccacaggtgtacaccctgcccccatcccgggatgagctgaccaagaaccaggtcagcctgacctgcctggtcaaaggcttctatcccagcgacatcgccgtggagtgggagagcaatgggcagccggagaacaactacaagaccacacctcccgtgctggactccgacggctccttcttcctctacagcaagctcaccgtggacaagagcaggtggcagcaggggaacgtcttctcatgctccgtgatgcatgaggctctgcacaaccactacacgcagaagagcctctccctgtccccgggtaaa

SEQ ID NO: 30 - protein, 227 aa, synthetic construct
  REGION 1..227: note = PFc 3
DKTHTCPLCPAPELLGGPSVFLFPPKPKDTLMISRTPEVTCVVVDVSHEDPEVKFNWYVDGVEVHNAKTKPREEQYNSTYRVVSVLTVRHQDWLNGKEYKCKVSNKALPAPIEKTISKAKGQPREPQVYTLPPSRDELTKNQVSLTCLVKGFYPSDIAVEWESNGQPENNYKTTPPVLDSDGSFFLYSKLTVDKSRWQQGNVFSCSVLHEALHSHYTQKSLSLSPGK

SEQ ID NO: 31 - protein, 227 aa, synthetic construct
  REGION 1..227: note = PFc 29
DKTHTCPPCPAPELLGGPSVFLFPPKPKDTLMISRTPEVTCVVVDVSHEDPEVKFNWYVDGVEVHNAKTKPREEQYNSTYRVVSVLTVLHRDWLNGKEYKCKVSNKALPAPIEKTISKAKGQPREPQVYTLPPSRDELTKNQVSLTCLVKGFYPSDIAVEWESNGQPENNYKTTPPVLDSDGSFFLYSKLTVDKSRWQQGNVFSCSVLHEALHNHYTQKSLSLSPGK

SEQ ID NO: 32 - protein, 227 aa, synthetic construct
  REGION 1..227: note = PFc 41
DKTHTCPPCPAPELLGGPSVFLFPPKPKDTLMISRTPEVTCVVVDVSHEDPEVKFNWYVDGVEVHNAKTKPREEQYNSTYRVVSVLTVGHQDWLNGKEYKCKVSNKALPAPIEKTISKAKGQPREPQVYTLPPSRDELTKNQVSLTCLVKGFYPSDIAVEWESNGQPENNYKTTPPVLDSDGSFFLYSKLTVDKSRWQQGNVFSCSVLHEALHNHYTQKSLSLSPGK

SEQ ID NO: 33 - protein, 227 aa, synthetic construct
  REGION 1..227: note = EFc 6
DKTHTCPLCPAPELLGGPSVFLFPPKPKDTLMISRTPEVTCVVMDVSHEDPEVKFNWYVDGVEVHNAKTKPREEQYNSTYRVVSVLTVLHQDWLNGKEYKCKVSNKALPAPIEKTISKAKGQPREPQVYTLPPSRDELTKNQVSLTCQVKGFYPSDIAVEWESNGQPDNNYKTTPPVLDSDGSFFLYSKLTVDKSRWQQGNDFSCSVLHEALHNHYTQKSLSLSSGK

SEQ ID NO: 34 - protein, 227 aa, synthetic construct
  REGION 1..227: note = EFc 29
DKTHTCPLCPAPELLGGPSVFLFPPKPKDTLMISRTPEVTCVVVDVSHEDPEVKFNWYVDGVEVHNAKTKPLEEQYNSTYRVVSVLTVLHQDWLNGKEYKCKVSNKALPAPIEKTISKAKGQPREPQVYTLPPSRDELAKNQVGLTCLVKGFYPSDIAVEWESNGQPENNYKTTPPVLDSDGSFFLYSKLTVDKSRWQQGNVFSCSVLHEALHNHYTQKSLSLSPGK

SEQ ID NO: 35 - protein, 227 aa, synthetic construct
  REGION 1..227: note = EFc 41
DKTHTCPLCPAPEFLGGPSVFLFPPKPKDTLMISRTPEVTCVVVDVSHDDPEVKFNWYVDGVEVHNAKTKPREEQYNSTYRVVSVLTVLHQDWLNGKEYKCKVSNKALPAPIEKTISKAKGLPREPQVYTLPPSRDELTKNQVSLTCLVKGFYPSDIAVEWESNGQPDNNYKTAPPVLDSDGSFFLYSKLTVDKSRWQQGNVFSCSVLHEALHNHYTQKSLSLSPGK

SEQ ID NO: 36 - protein, 227 aa, synthetic construct
  REGION 1..227: note = EFc 82
DKTHTCPPCQAPELLGGPSVFLYPPEPKDTLMISRTPEVTCVVVDVSHEDPEVKFNWYVDGVEVHNAKTKPREEQYNSTYRVVSVLTVLHQDWLNGKEYKCKVSNKALPAPIEKTISKAKGQPREPQVYTLPPSRDELTKSQVSLTCLVKGFYPSDIAVEWESIGQPENNYKTTPPVLDSDGSFFLYSKLTVDKSRWQQGNVFSCSVLHEALHNHYTQKSLSLSPGK

SEQ ID NO: 37 - protein, 227 aa, synthetic construct
  REGION 1..227: note = EFc 88
DKTHTCPPCSAPELLGGPSVFLFPPKPKDTLMISRTPEVTCVVVDVSHEDPEVKFNWYVDGVEVHNAKTKPREELYNSTYRVVSVLTVLHQDWLNGKEYMCKVSNKALPAPIEKTISKAKGQPREPQVYTLPPSREELTKNQVSLTCLVKGFYPSDIAVEWESNGQPENNYKTTPPVLDSDGSFILYSKLTVDKSRWQQGNVFSCSVLHEALHNHYTQKSLSLSPGK